European Patent Application EP 4 663 770 A1, published December 17, 2025. Title: Method for detecting mutant nucleic acid. Applicant: Seoul National University R&DB Foundation. Application KR 10-2023-0016723, filed February 8, 2023. The sequence listing filed with the application follows.

SEQUENCE LISTING (36 sequences)

SEQ ID NO: 1 - DNA, 114 bp, Homo sapiens
  source 1..114: mol_type = other DNA
aggcctgctgaaaatgactgaatataaacttgtggtagttggagctggtggcgtaggcaagagtgccttgacgatacagctaattcagaatcattttgtggacgaatatgatcc

SEQ ID NO: 2 - DNA, 114 bp, Homo sapiens
  source 1..114: mol_type = other DNA
aggcctgctgaaaatgactgaatataaacttgtggtagttggagctgatggcgtaggcaagagtgccttgacgatacagctaattcagaatcattttgtggacgaatatgatcc

SEQ ID NO: 3 - DNA, 114 bp, Homo sapiens
  source 1..114: mol_type = other DNA
aggcctgctgaaaatgactgaatataaacttgtggtagttggagcttgtggcgtaggcaagagtgccttgacgatacagctaattcagaatcattttgtggacgaatatgatcc

SEQ ID NO: 4 - DNA, 114 bp, Homo sapiens
  source 1..114: mol_type = other DNA
aggcctgctgaaaatgactgaatataaacttgtggtagttggagctgttggcgtaggcaagagtgccttgacgatacagctaattcagaatcattttgtggacgaatatgatcc

SEQ ID NO: 5 - DNA, 25 bp, synthetic construct
  source 1..25: mol_type = other DNA
  modified_base 1: mod_base = OTHER; note = biotinylated
aggcctgctgaaaatgactgaatat

SEQ ID NO: 6 - DNA, 20 bp, synthetic construct
  source 1..20: mol_type = other DNA
  modified_base 1: mod_base = OTHER; note = phosphorylated
ggatcatattcgtccacaaa

SEQ ID NO: 7 - DNA, 35 bp, synthetic construct
  source 1..35: mol_type = other DNA
ccacaagtttatattcagtcattttcagcaggcct

SEQ ID NO: 8 - DNA, 59 bp, synthetic construct
  source 1..59: mol_type = other DNA
ggatcatattcgtccacaaaatgattctgaattagctgtatcgtcaaggcactcttgcc

SEQ ID NO: 9 - DNA, 21 bp, synthetic construct
  source 1..21: mol_type = other DNA
  modified_base 1: mod_base = OTHER; note = phosphorylated
  modified_base 18: mod_base = OTHER; note = amine-modified
ccaccagctcgttgatgtaat

SEQ ID NO: 10 - DNA, 21 bp, synthetic construct
  source 1..21: mol_type = other DNA
  modified_base 1: mod_base = OTHER; note = phosphorylated
  modified_base 18: mod_base = OTHER; note = amine-modified
ccatcagctcgttgatgtaat

SEQ ID NO: 11 - DNA, 21 bp, synthetic construct
  source 1..21: mol_type = other DNA
  modified_base 1: mod_base = OTHER; note = phosphorylated
  modified_base 18: mod_base = OTHER; note = amine-modified
ccacaagctcgttgatgtaat

SEQ ID NO: 12 - DNA, 21 bp, synthetic construct
  source 1..21: mol_type = other DNA
  modified_base 1: mod_base = OTHER; note = phosphorylated
  modified_base 18: mod_base = OTHER; note = amine-modified
ccaacagctcgttgatgtaat

SEQ ID NO: 13 - DNA, 111 bp, Homo sapiens
  source 1..111: mol_type = other DNA
cttcatgaagacctcacagtaaaaataggtgattttggtctagctacagtgaaatctcgatggagtgggtcccatcagtttgaacagttgtctggatccattttgtggatg

SEQ ID NO: 14 - DNA, 111 bp, Homo sapiens
  source 1..111: mol_type = other DNA
cttcatgaagacctcacagtaaaaataggtgattttggtctagctacaaagaaatctcgatggagtgggtcccatcagtttgaacagttgtctggatccattttgtggatg

SEQ ID NO: 15 - DNA, 111 bp, Homo sapiens
  source 1..111: mol_type = other DNA
cttcatgaagacctcacagtaaaaataggtgattttggtctagctacagagaaatctcgatggagtgggtcccatcagtttgaacagttgtctggatccattttgtggatg

SEQ ID NO: 16 - DNA, 20 bp, synthetic construct
  source 1..20: mol_type = other DNA
  modified_base 1: mod_base = OTHER; note = biotinylated
cttcatgaagacctcacagt

SEQ ID NO: 17 - DNA, 20 bp, synthetic construct
  source 1..20: mol_type = other DNA
  modified_base 1: mod_base = OTHER; note = phosphorylated
catccacaaaatggatccag

SEQ ID NO: 18 - DNA, 32 bp, synthetic construct
  source 1..32: mol_type = other DNA
tcacctatttttactgtgaggtcttcatgaag

SEQ ID NO: 19 - DNA, 54 bp, synthetic construct
  source 1..54: mol_type = other DNA
catccacaaaatggatccagacaactgttcaaactgatgggacccactccatcg

SEQ ID NO: 20 - DNA, 21 bp, synthetic construct
  source 1..21: mol_type = other DNA
  modified_base 1: mod_base = OTHER; note = phosphorylated
  modified_base 18: mod_base = OTHER; note = amine-modified
ttcactgtagcatatattatt

SEQ ID NO: 21 - DNA, 21 bp, synthetic construct
  source 1..21: mol_type = other DNA
  modified_base 1: mod_base = OTHER; note = phosphorylated
  modified_base 18: mod_base = OTHER; note = amine-modified
ttctttgtagctaatattatt

SEQ ID NO: 22 - DNA, 21 bp, synthetic construct
  source 1..21: mol_type = other DNA
  modified_base 1: mod_base = OTHER; note = phosphorylated
  modified_base 18: mod_base = OTHER; note = amine-modified
ttctctgtagcattatttatt

SEQ ID NO: 23 - DNA, 34 bp, synthetic construct
  source 1..34: mol_type = other DNA
cttgtggtagttggagctggtggcgtaggcaaga

SEQ ID NO: 24 - DNA, 34 bp, synthetic construct
  source 1..34: mol_type = other DNA
tcttgcctacgccaccagctccaactaccacaag

SEQ ID NO: 25 - DNA, 34 bp, synthetic construct
  source 1..34: mol_type = other DNA
cttgtggtagttggagctgatggcgtaggcaaga

SEQ ID NO: 26 - DNA, 34 bp, synthetic construct
  source 1..34: mol_type = other DNA
tcttgcctacgccatcagctccaactaccacaag

SEQ ID NO: 27 - DNA, 34 bp, synthetic construct
  source 1..34: mol_type = other DNA
cttgtggtagttggagcttgtggcgtaggcaaga

SEQ ID NO: 28 - DNA, 34 bp, synthetic construct
  source 1..34: mol_type = other DNA
tcttgcctacgccacaagctccaactaccacaag

SEQ ID NO: 29 - DNA, 34 bp, synthetic construct
  source 1..34: mol_type = other DNA
cttgtggtagttggagctgttggcgtaggcaaga

SEQ ID NO: 30 - DNA, 34 bp, synthetic construct
  source 1..34: mol_type = other DNA
tcttgcctacgccaacagctccaactaccacaag

SEQ ID NO: 31 - DNA, 34 bp, synthetic construct
  source 1..34: mol_type = other DNA
ggtgattttggtctagctacagtgaaatctcgat

SEQ ID NO: 32 - DNA, 34 bp, synthetic construct
  source 1..34: mol_type = other DNA
atcgagatttcactgtagctagaccaaaatcacc

SEQ ID NO: 33 - DNA, 34 bp, synthetic construct
  source 1..34: mol_type = other DNA
ggtgattttggtctagctacaaagaaatctcgat

SEQ ID NO: 34 - DNA, 34 bp, synthetic construct; identical to SEQ ID NO: 32
  source 1..34: mol_type = other DNA

SEQ ID NO: 35 - DNA, 34 bp, synthetic construct
  source 1..34: mol_type = other DNA
ggtgattttggtctagctacagagaaatctcgat

SEQ ID NO: 36 - DNA, 34 bp, synthetic construct; identical to SEQ ID NO: 32
  source 1..34: mol_type = other DNA